European Patent Application EP 4 553 159 A1, published May 14, 2025. Title: Steviol glycoside biosynthesis enzyme variant and use thereof. Applicant: SUNTORY HOLDINGS LIMITED. The sequence listing filed with the application follows.

SEQUENCE LISTING (18 sequences)

SEQ ID NO: 1 - DNA, 1458 bp, synthetic construct
  source 1..1458: mol_type = other DNA
atgtacaacgttacttatcatcaaaattcaaaagcaatggctaccagtgactccatagttgacgaccgtaagcagcttcatgttgcgacgttcccatggcttgctttcggtcacatcctcccttaccttcagctttcgaaattgatagctgaaaagggtcacaaagtctcgtttctttctaccaccagaaacattcaacgtctctcttctcatatctcgccactcataaatgttgttcaactcacacttccacgtgtccaagagctgccggaggatgcagaggcgaccactgacgtccaccctgaagatattccatatctcaagaaggcttctgatggtcttcaaccggaggtcacccggtttctagaacaacactctccggactggattatttatgattatactcactactggttgccatccatcgcggctagcctcggtatctcacgagcccacttctccaccaccactccatgggccattgcttatatgggaccctcagctgacgccatgataaatggttcagatggtcgaaccacggttgaggatctcacgacaccgcccaagtggtttccctttccgaccaaagtatgctggcggaagcatgatcttgcccgactggtgccttacaaagctccggggatatctgatggataccgtatggggctggttcttaagggatctgattgtttgctttccaaatgttaccatgagtttggaactcaatggctacctcttttggagacactacaccaagtaccggtggttccggtgggattactgccaccggaaatacccggagacgagaaagatgaaacatgggtgtcaatcaagaaatggctcgatggtaaacaaaaaggcagtgtggtgtacgttgcattaggaagcgaggttttggtgagccaaaccgaggttgttgagttagcattgggtctcgagctttctgggttgccatttgtttgggcttatagaaaaccaaaaggtcccgcgaagtcagactcggtggagttgccagacgggttcgtggaacgaactcgtgaccgtgggttggtctggacgagttgggcacctcagttacgaatactgagccatgagtcggtttgtggtttcttgactcattgtggttctggatcaattgtggaagggctaatgtttggtcaccctctaatcatgctaccgatttttggggaccaacctctgaatgctcgattactggaggacaaacaggtgggaatcgagataccaagaaatgaggaagatggttgcttgaccaaggagtcggttgctagatcactgaggtccgttgttgtggaaaaagaaggggagatctacaaggcgaacgcgagggagctgagtaaaatctataacgacactaaggttgaaaaagaatatgtaagccaattcgtagactatttggaaaagaatgcgcgtgcggttgccatcgatcatgagagttaa

SEQ ID NO: 2 - protein, 485 aa, synthetic construct
MYNVTYHQNSKAMATSDSIVDDRKQLHVATFPWLAFGHILPYLQLSKLIAEKGHKVSFLSTTRNIQRLSSHISPLINVVQLTLPRVQELPEDAEATTDVHPEDIPYLKKASDGLQPEVTRFLEQHSPDWIIYDYTHYWLPSIAASLGISRAHFSTTTPWAIAYMGPSADAMINGSDGRTTVEDLTTPPKWFPFPTKVCWRKHDLARLVPYKAPGISDGYRMGLVLKGSDCLLSKCYHEFGTQWLPLLETLHQVPVVPVGLLPPEIPGDEKDETWVSIKKWLDGKQKGSVVYVALGSEVLVSQTEVVELALGLELSGLPFVWAYRKPKGPAKSDSVELPDGFVERTRDRGLVWTSWAPQLRILSHESVCGFLTHCGSGSIVEGLMFGHPLIMLPIFGDQPLNARLLEDKQVGIEIPRNEEDGCLTKESVARSLRSVVVEKEGEIYKANARELSKIYNDTKVEKEYVSQFVDYLEKNARAVAIDHES

SEQ ID NO: 3 - DNA, 1458 bp, synthetic construct
  source 1..1458: mol_type = other DNA
atgtacaacgttacttatcatcaaaattcaaaagcaatggctaccagtgactccatagttgacgaccgtaagcagcttcatgttgcgacgttcccatggcttgctttcggtcacatcctccctttccttcagctttcgaaattgatagctgaaaagggtcacaaagtctcgtttctttctaccaccagaaacattcaacgtctctcttctcatatctcgccactcataaatgttgttcaactcacacttccacgtgtccaagagctgccggaggatgcagaggcgaccactgacgtccaccctgaagatattccatatctcaagaaggcttctgatggtcttcaaccggaggtcacccggtttctagaacaacactctccggactggattatttatgattatactcactactggttgccatccatcgcggctagcctcggtatctcacgagcccacttctccaccaccactccatgggccattgcttatatgggaccctcagctgacgccatgataaatggttcagatggtcgaaccacggttgaggatctcacgacaccgcccaagtggtttccctttccgaccaaagtatgctggcggaagcatgatcttgcccgactggtgccttacaaagctccggggatatctgatggataccgtatggggctggttcttaagggatctgattgtttgctttccaaatgttaccatgagtttggaactcaatggctacctcttttggagacactacaccaagtaccggtggttccggtgggattactgccaccggaaatacccggagacgagaaagatgaaacatgggtgtcaatcaagaaatggctcgatggtaaacaaaaaggcagtgtggtgtacgttgcattaggaagcgaggttttggtgagccaaaccgaggttgttgagttagcattgggtctcgagctttctgggttgccatttgtttgggcttatagaaaaccaaaaggtcccgcgaagtcagactcggtggagttgccagacgggttcgtggaacgaactcgtgaccgtgggttggtctggacgagttgggcacctcagttacgaatactgagccatgagtcggtttgtggtttcttgactcattgtggttctggatcaattgtggaagggctaatgtttggtcaccctctaatcatgctaccgatttttggggaccaacctctgaatgctcgattactggaggacaaacaggtgggaatcgagataccaagaaatgaggaagatggttgcttgaccaaggagtcggttgctagatcactgaggtccgttgttgtggaaaaagaaggggagatctacaaggcgaacgcgagggagctgagtaaaatctataacgacactaaggttgaaaaagaatatgtaagccaattcgtagactatttggaaaagaatgcgcgtgcggttgccatcgatcatgagagttaa

SEQ ID NO: 4 - protein, 485 aa, synthetic construct
MYNVTYHQNSKAMATSDSIVDDRKQLHVATFPWLAFGHILPFLQLSKLIAEKGHKVSFLSTTRNIQRLSSHISPLINVVQLTLPRVQELPEDAEATTDVHPEDIPYLKKASDGLQPEVTRFLEQHSPDWIIYDYTHYWLPSIAASLGISRAHFSTTTPWAIAYMGPSADAMINGSDGRTTVEDLTTPPKWFPFPTKVCWRKHDLARLVPYKAPGISDGYRMGLVLKGSDCLLSKCYHEFGTQWLPLLETLHQVPVVPVGLLPPEIPGDEKDETWVSIKKWLDGKQKGSVVYVALGSEVLVSQTEVVELALGLELSGLPFVWAYRKPKGPAKSDSVELPDGFVERTRDRGLVWTSWAPQLRILSHESVCGFLTHCGSGSIVEGLMFGHPLIMLPIFGDQPLNARLLEDKQVGIEIPRNEEDGCLTKESVARSLRSVVVEKEGEIYKANARELSKIYNDTKVEKEYVSQFVDYLEKNARAVAIDHES

SEQ ID NO: 5 - DNA, 1458 bp, Stevia rebaudiana
  source 1..1458: mol_type = other DNA
atgtacaacgttacttatcatcaaaattcaaaagcaatggctaccagtgactccatagttgacgaccgtaagcagcttcatgttgcgacgttcccatggcttgctttcggtcacatcctcccttaccttcagctttcgaaattgatagctgaaaagggtcacaaagtctcgtttctttctaccaccagaaacattcaacgtctctcttctcatatctcgccactcataaatgttgttcaactcacacttccacgtgtccaagagctgccggaggatgcagaggcgaccactgacgtccaccctgaagatattccatatctcaagaaggcttctgatggtcttcaaccggaggtcacccggtttctagaacaacactctccggactggattatttatgattatactcactactggttgccatccatcgcggctagcctcggtatctcacgagcccacttctccgtcaccactccatgggccattgcttatatgggaccctcagctgacgccatgataaatggttcagatggtcgaaccacggttgaggatctcacgacaccgcccaagtggtttccctttccgaccaaagtatgctggcggaagcatgatcttgcccgactggtgccttacaaagctccggggatatctgatggataccgtatggggctggttcttaagggatctgattgtttgctttccaaatgttaccatgagtttggaactcaatggctacctcttttggagacactacaccaagtaccggtggttccggtgggattactgccaccggaaatacccggagacgagaaagatgaaacatgggtgtcaatcaagaaatggctcgatggtaaacaaaaaggcagtgtggtgtacgttgcattaggaagcgaggttttggtgagccaaaccgaggttgttgagttagcattgggtctcgagctttctgggttgccatttgtttgggcttatagaaaaccaaaaggtcccgcgaagtcagactcggtggagttgccagacgggttcgtggaacgaactcgtgaccgtgggttggtctggacgagttgggcacctcagttacgaatactgagccatgagtcggtttgtggtttcttgactcattgtggttctggatcaattgtggaagggctaatgtttggtcaccctctaatcatgctaccgatttttggggaccaacctctgaatgctcgattactggaggacaaacaggtgggaatcgagataccaagaaatgaggaagatggttgcttgaccaaggagtcggttgctagatcactgaggtccgttgttgtggaaaaagaaggggagatctacaaggcgaacgcgagggagctgagtaaaatctataacgacactaaggttgaaaaagaatatgtaagccaattcgtagactatttggaaaagaatgcgcgtgcggttgccatcgatcatgagagttaa

SEQ ID NO: 6 - protein, 485 aa, Stevia rebaudiana
MYNVTYHQNSKAMATSDSIVDDRKQLHVATFPWLAFGHILPYLQLSKLIAEKGHKVSFLSTTRNIQRLSSHISPLINVVQLTLPRVQELPEDAEATTDVHPEDIPYLKKASDGLQPEVTRFLEQHSPDWIIYDYTHYWLPSIAASLGISRAHFSVTTPWAIAYMGPSADAMINGSDGRTTVEDLTTPPKWFPFPTKVCWRKHDLARLVPYKAPGISDGYRMGLVLKGSDCLLSKCYHEFGTQWLPLLETLHQVPVVPVGLLPPEIPGDEKDETWVSIKKWLDGKQKGSVVYVALGSEVLVSQTEVVELALGLELSGLPFVWAYRKPKGPAKSDSVELPDGFVERTRDRGLVWTSWAPQLRILSHESVCGFLTHCGSGSIVEGLMFGHPLIMLPIFGDQPLNARLLEDKQVGIEIPRNEEDGCLTKESVARSLRSVVVEKEGEIYKANARELSKIYNDTKVEKEYVSQFVDYLEKNARAVAIDHES

SEQ ID NO: 7 - DNA, 1383 bp, Stevia rebaudiana
  source 1..1383: mol_type = other DNA
atggcggaacaacaaaagatcaagaaatcaccacacgttctactcatcccattccctttacaaggccatataaaccctttcatccagtttggcaaacgattaatctccaaaggtgtcaaaacaacacttgttaccaccatccacaccttaaactcaaccctaaaccacagtaacaccaccaccacctccatcgaaatccaagcaatttccgatggttgtgatgaaggcggttttatgagtgcaggagaatcatatttggaaacattcaaacaagttgggtctaaatcactagctgacttaatcaagaagcttcaaagtgaaggaaccacaattgatgcaatcatttatgattctatgactgaatgggttttagatgttgcaattgagtttggaatcgatggtggttcgtttttcactcaagcttgtgttgtaaacagcttatattatcatgttcataagggtttgatttctttgccattgggtgaaactgtttcggttcctggatttccagagcttcaacggtgggagacaccgttaattttgcagaatcatgagcaaatacagagcccttggtctcagatgttgtttggtcagtttgctaatattgatcaagcacgttgggtcttcacaaatagtttttacaagctcgaggaagaggtaatagagtggacgagaaagatatggaacttgaaggtaatcgggccaacacttccatccatgtaccttgacaaacgacttgatgatgataaagataacggatttaatctctacaaagcaaaccatcatgagtgcatgaactggttagacgataagccaaaggaatcagttgtttacgtagcatttggtagcctggtgaaacatggacccgaacaagtggaagaaatcacacgggctttaatagatagtgatgtcaacttcttgtgggttatcaaacataaagaagagggaaagctcccagaaaatctttcggaagtaataaaaaccggaaagggtttgattgtagcatggtgcaaacaattggatgtgttagcacacgaatcagtaggatgctttgttacacattgtgggttcaactcaactcttgaagcaataagtcttggagtccccgttgttgcaatgcctcaattttcggatcaaactacaaatgccaagcttctagatgaaattttgggtgttggagttagagttaaggctgatgagaatgggatagtgagaagaggaaatcttgcgtcatgtattaagatgattatggaggaggaaagaggagtaataatccgaaagaatgcggtaaaatggaaggatttggctaaagtagccgttcatgaaggtggtagctcagacaatgatattgtcgaatttgtaagtgagctaattaaggcttaa

SEQ ID NO: 8 - protein, 460 aa, Stevia rebaudiana
MAEQQKIKKSPHVLLIPFPLQGHINPFIQFGKRLISKGVKTTLVTTIHTLNSTLNHSNTTTTSIEIQAISDGCDEGGFMSAGESYLETFKQVGSKSLADLIKKLQSEGTTIDAIIYDSMTEWVLDVAIEFGIDGGSFFTQACVVNSLYYHVHKGLISLPLGETVSVPGFPELQRWETPLILQNHEQIQSPWSQMLFGQFANIDQARWVFTNSFYKLEEEVIEWTRKIWNLKVIGPTLPSMYLDKRLDDDKDNGFNLYKANHHECMNWLDDKPKESVVYVAFGSLVKHGPEQVEEITRALIDSDVNFLWVIKHKEEGKLPENLSEVIKTGKGLIVAWCKQLDVLAHESVGCFVTHCGFNSTLEAISLGVPVVAMPQFSDQTTNAKLLDEILGVGVRVKADENGIVRRGNLASCIKMIMEEERGVIIRKNAVKWKDLAKVAVHEGGSSDNDIVEFVSELIKA

SEQ ID NO: 9 - DNA, 1377 bp, Stevia rebaudiana
  source 1..1377: mol_type = other DNA
atggaaaataaaacggagaccaccgttcgccggcgccggagaataatattattcccggtaccatttcaaggccacattaacccaattcttcagctagccaatgtgttgtactctaaaggattcagtatcaccatctttcacaccaacttcaacaaacccaaaacatctaattaccctcacttcactttcagattcatcctcgacaacgacccacaagacgaacgcatttccaatctaccgactcatggtccgctcgctggtatgcggattccgattatcaacgaacacggagctgacgaattacgacgcgaactggaactgttgatgttagcttctgaagaagatgaagaggtatcgtgtttaatcacggatgctctttggtacttcgcgcaatctgttgctgacagtcttaacctccgaccgcttgttttgatgacaagcagcttgtttaattttcatgcacatgtttcacttcctcagtttgatgagcttggttacctcgatcctgatgacaaaacccgtttggaagaacaagcgagtgggtttcctatgctaaaagtgaaagacatcaagtctgcgtattcgaactggcaaatactcaaagagatattagggaagatgataaaacaaacaaaagcatcttcaggagtcatctggaactcatttaaggaactcgaagagtctgagctcgaaactgttatccgtgagatcccggctccaagtttcttgataccactccccaagcatttgacagcctcttccagcagcttactagaccacgatcgaaccgtttttcaatggttagaccaacaaccgccaagttcggtactgtatgttagttttggtagtactagtgaagtggatgagaaagatttcttggaaatagctcgtgggttggttgatagcaagcagtcgtttttatgggtggttcgacctgggtttgtcaagggttcgacgtgggtcgaaccgttgccagatgggttcttgggtgaaagaggacgtattgtgaaatgggttccacagcaagaagtgctagctcatggagcaataggcgcattctggactcatagcggatggaactctacgttggaaagcgtttgtgaaggtgttcctatgattttctcggattttgggctcgatcaaccgttgaatgctagatacatgagtgatgttttgaaggtaggggtgtatttggaaaatgggtgggaaagaggagagatagcaaatgcaataagaagagttatggtggatgaagaaggagaatacattagacagaatgcaagagttttgaaacaaaaggcagatgtttctttgatgaagggtggttcgtcttacgaatcattagagtctctagtttcttacatttcatcgttgtaa

SEQ ID NO: 10 - protein, 458 aa, Stevia rebaudiana
MENKTETTVRRRRRIILFPVPFQGHINPILQLANVLYSKGFSITIFHTNFNKPKTSNYPHFTFRFILDNDPQDERISNLPTHGPLAGMRIPIINEHGADELRRELELLMLASEEDEEVSCLITDALWYFAQSVADSLNLRPLVLMTSSLFNFHAHVSLPQFDELGYLDPDDKTRLEEQASGFPMLKVKDIKSAYSNWQILKEILGKMIKQTKASSGVIWNSFKELEESELETVIREIPAPSFLIPLPKHLTASSSSLLDHDRTVFQWLDQQPPSSVLYVSFGSTSEVDEKDFLEIARGLVDSKQSFLWVVRPGFVKGSTWVEPLPDGFLGERGRIVKWVPQQEVLAHGAIGAFWTHSGWNSTLESVCEGVPMIFSDFGLDQPLNARYMSDVLKVGVYLENGWERGEIANAIRRVMVDEEGEYIRQNARVLKQKADVSLMKGGSSYESLESLVSYISSL

SEQ ID NO: 11 - DNA, 1446 bp, Stevia rebaudiana
  source 1..1446: mol_type = other DNA
atggatgcaatggctacaactgagaagaaaccacacgtcatcttcataccatttccagcacaaagccacattaaagccatgctcaaactagcacaacttctccaccacaaaggactccagataaccttcgtcaacaccgacttcatccacaaccagtttcttgaatcatcgggcccacattgtttggacggttcaccgggtttccggttcgaaaccatcccggatggtgtttctcacagtccggaagcgagcatcccaatcagagaatcactcttgagatccattgaaaccaacttcttggatcgtttcattgatcttgtaaccaaacttccggatcctccgacttgtattatctcagatgggttcttgtcggttttcacaattgacgctgcaaaaaagcttggaattccggtcatgatgtattggacacttgctgcctgtgggttcatgggtttttaccatattcattctctcattgagaaaggatttgcaccacttaaagatgcaagttacttgacaaatgggtatttggacaccgtcattgattgggttccgggaatggaaggcatccgtctcaaggatttcccgctggactggagcactgacctcaatgacaaagttttgatgttcactacagaagctcctcaaaggtcacacaaggtttcacatcatattttccacacgttcgatgagttggagcctagtattataaaaactttgtcattgaggtataatcacatttacaccatcggcccactgcaattacttcttgatcaaatacccgaagagaaaaagcaaactggaattacgagtctccatggatacagtttagtaaaagaagaaccagagtgtttccagtggcttcagtctaaagaaccaaattccgtcgtttatgtaaattttggaagtactacagtaatgtctttagaagacatgacggaatttggttggggacttgctaatagcaaccattatttcctttggatcatccgatcaaacttggtgataggggaaaatgcagttttgccccctgaacttgaggaacatataaagaaaagaggctttattgctagctggtgttcacaagaaaaggtcttgaagcacccttcggttggagggttcttgactcattgtgggtggggatcgaccatcgagagcttgtctgctggggtgccaatgatatgctggccttattcgtgggaccagctgaccaactgtaggtatatatgcaaagaatgggaggttgggctcgagatgggaaccaaagtgaaacgagatgaagtcaagaggcttgtacaagagttgatgggagaaggaggtcacaaaatgaggaacaaggctaaagattggaaagaaaaggctcgcattgcaatagctcctaacggttcatcttctttgaacatagacaaaatggtcaaggaaatcaccgtgctagcaagaaactag

SEQ ID NO: 12 - protein, 481 aa, Stevia rebaudiana
MDAMATTEKKPHVIFIPFPAQSHIKAMLKLAQLLHHKGLQITFVNTDFIHNQFLESSGPHCLDGSPGFRFETIPDGVSHSPEASIPIRESLLRSIETNFLDRFIDLVTKLPDPPTCIISDGFLSVFTIDAAKKLGIPVMMYWTLAACGFMGFYHIHSLIEKGFAPLKDASYLTNGYLDTVIDWVPGMEGIRLKDFPLDWSTDLNDKVLMFTTEAPQRSHKVSHHIFHTFDELEPSIIKTLSLRYNHIYTIGPLQLLLDQIPEEKKQTGITSLHGYSLVKEEPECFQWLQSKEPNSVVYVNFGSTTVMSLEDMTEFGWGLANSNHYFLWIIRSNLVIGENAVLPPELEEHIKKRGFIASWCSQEKVLKHPSVGGFLTHCGWGSTIESLSAGVPMICWPYSWDQLTNCRYICKEWEVGLEMGTKVKRDEVKRLVQELMGEGGHKMRNKAKDWKEKARIAIAPNGSSSLNIDKMVKEITVLARN

SEQ ID NO: 13 - DNA, 1478 bp, synthetic construct
  source 1..1478: mol_type = other DNA
gcggccgcaaaaatgtacaacgttacttatcatcaaaattcaaaagcaatggctaccagtgactccatagttgacgaccgtaagcagcttcatgttgcgacgttcccatggcttgctttcggtcacatcctcccttaccttcagctttcgaaattgatagctgaaaagggtcacaaagtctcgtttctttctaccaccagaaacattcaacgtctctcttctcatatctcgccactcataaatgttgttcaactcacacttccacgtgtccaagagctgccggaggatgcagaggcgaccactgacgtccaccctgaagatattccatatctcaagaaggcttctgatggtcttcaaccggaggtcacccggtttctagaacaacactctccggactggattatttatgattatactcactactggttgccatccatcgcggctagcctcggtatctcacgagcccacttctccgtcaccactccatgggccattgcttatatgggaccctcagctgacgccatgataaatggttcagatggtcgaaccacggttgaggatctcacgacaccgcccaagtggtttccctttccgaccaaagtatgctggcggaagcatgatcttgcccgactggtgccttacaaagctccggggatatctgatggataccgtatggggctggttcttaagggatctgattgtttgctttccaaatgttaccatgagtttggaactcaatggctacctcttttggagacactacaccaagtaccggtggttccggtgggattactgccaccggaaatacccggagacgagaaagatgaaacatgggtgtcaatcaagaaatggctcgatggtaaacaaaaaggcagtgtggtgtacgttgcattaggaagcgaggttttggtgagccaaaccgaggttgttgagttagcattgggtctcgagctttctgggttgccatttgtttgggcttatagaaaaccaaaaggtcccgcgaagtcagactcggtggagttgccagacgggttcgtggaacgaactcgtgaccgtgggttggtctggacgagttgggcacctcagttacgaatactgagccatgagtcggtttgtggtttcttgactcattgtggttctggatcaattgtggaagggctaatgtttggtcaccctctaatcatgctaccgatttttggggaccaacctctgaatgctcgattactggaggacaaacaggtgggaatcgagataccaagaaatgaggaagatggttgcttgaccaaggagtcggttgctagatcactgaggtccgttgttgtggaaaaagaaggggagatctacaaggcgaacgcgagggagctgagtaaaatctataacgacactaaggttgaaaaagaatatgtaagccaattcgtagactatttggaaaagaatgcgcgtgcggttgccatcgatcatgagagttaattaattaa

SEQ ID NO: 14 - DNA, 1478 bp, synthetic construct
  source 1..1478: mol_type = other DNA
gcggccgcaaaaatgtacaacgttacttatcatcaaaattcaaaagcaatggctaccagtgactccatagttgacgaccgtaagcagcttcatgttgcgacgttcccatggcttgctttcggtcacatcctcccttaccttcagctttcgaaattgatagctgaaaagggtcacaaagtctcgtttctttctaccaccagaaacattcaacgtctctcttctcatatctcgccactcataaatgttgttcaactcacacttccacgtgtccaagagctgccggaggatgcagaggcgaccactgacgtccaccctgaagatattccatatctcaagaaggcttctgatggtcttcaaccggaggtcacccggtttctagaacaacactctccggactggattatttatgattatactcactactggttgccatccatcgcggctagcctcggtatctcacgagcccacttctccaccaccactccatgggccattgcttatatgggaccctcagctgacgccatgataaatggttcagatggtcgaaccacggttgaggatctcacgacaccgcccaagtggtttccctttccgaccaaagtatgctggcggaagcatgatcttgcccgactggtgccttacaaagctccggggatatctgatggataccgtatggggctggttcttaagggatctgattgtttgctttccaaatgttaccatgagtttggaactcaatggctacctcttttggagacactacaccaagtaccggtggttccggtgggattactgccaccggaaatacccggagacgagaaagatgaaacatgggtgtcaatcaagaaatggctcgatggtaaacaaaaaggcagtgtggtgtacgttgcattaggaagcgaggttttggtgagccaaaccgaggttgttgagttagcattgggtctcgagctttctgggttgccatttgtttgggcttatagaaaaccaaaaggtcccgcgaagtcagactcggtggagttgccagacgggttcgtggaacgaactcgtgaccgtgggttggtctggacgagttgggcacctcagttacgaatactgagccatgagtcggtttgtggtttcttgactcattgtggttctggatcaattgtggaagggctaatgtttggtcaccctctaatcatgctaccgatttttggggaccaacctctgaatgctcgattactggaggacaaacaggtgggaatcgagataccaagaaatgaggaagatggttgcttgaccaaggagtcggttgctagatcactgaggtccgttgttgtggaaaaagaaggggagatctacaaggcgaacgcgagggagctgagtaaaatctataacgacactaaggttgaaaaagaatatgtaagccaattcgtagactatttggaaaagaatgcgcgtgcggttgccatcgatcatgagagttaattaattaa

SEQ ID NO: 15 - DNA, 1478 bp, synthetic construct
  source 1..1478: mol_type = other DNA
gcggccgcaaaaatgtacaacgttacttatcatcaaaattcaaaagcaatggctaccagtgactccatagttgacgaccgtaagcagcttcatgttgcgacgttcccatggcttgctttcggtcacatcctccctttccttcagctttcgaaattgatagctgaaaagggtcacaaagtctcgtttctttctaccaccagaaacattcaacgtctctcttctcatatctcgccactcataaatgttgttcaactcacacttccacgtgtccaagagctgccggaggatgcagaggcgaccactgacgtccaccctgaagatattccatatctcaagaaggcttctgatggtcttcaaccggaggtcacccggtttctagaacaacactctccggactggattatttatgattatactcactactggttgccatccatcgcggctagcctcggtatctcacgagcccacttctccaccaccactccatgggccattgcttatatgggaccctcagctgacgccatgataaatggttcagatggtcgaaccacggttgaggatctcacgacaccgcccaagtggtttccctttccgaccaaagtatgctggcggaagcatgatcttgcccgactggtgccttacaaagctccggggatatctgatggataccgtatggggctggttcttaagggatctgattgtttgctttccaaatgttaccatgagtttggaactcaatggctacctcttttggagacactacaccaagtaccggtggttccggtgggattactgccaccggaaatacccggagacgagaaagatgaaacatgggtgtcaatcaagaaatggctcgatggtaaacaaaaaggcagtgtggtgtacgttgcattaggaagcgaggttttggtgagccaaaccgaggttgttgagttagcattgggtctcgagctttctgggttgccatttgtttgggcttatagaaaaccaaaaggtcccgcgaagtcagactcggtggagttgccagacgggttcgtggaacgaactcgtgaccgtgggttggtctggacgagttgggcacctcagttacgaatactgagccatgagtcggtttgtggtttcttgactcattgtggttctggatcaattgtggaagggctaatgtttggtcaccctctaatcatgctaccgatttttggggaccaacctctgaatgctcgattactggaggacaaacaggtgggaatcgagataccaagaaatgaggaagatggttgcttgaccaaggagtcggttgctagatcactgaggtccgttgttgtggaaaaagaaggggagatctacaaggcgaacgcgagggagctgagtaaaatctataacgacactaaggttgaaaaagaatatgtaagccaattcgtagactatttggaaaagaatgcgcgtgcggttgccatcgatcatgagagttaattaattaa

SEQ ID NO: 16 - DNA, 1457 bp, synthetic construct
  source 1..1457: mol_type = other DNA
agatctatggatgcaatggctacaactgagaagaaaccacacgtcatcttcataccatttccagcacaaagccacattaaagccatgctcaaactagcacaacttctccaccacaaaggactccagataaccttcgtcaacaccgacttcatccacaaccagtttcttgaatcatcgggcccacattgtttggacggttcaccgggtttccggttcgaaaccatcccggatggtgtttctcacagtccggaagcgagcatcccaatcagagaatcactcttgagatccattgaaaccaacttcttggatcgtttcattgatcttgtaaccaaacttccggatcctccgacttgtattatctcagatgggttcttgtcggttttcacaattgacgctgcaaaaaagcttggaattccggtcatgatgtattggacacttgctgcctgtgggttcatgggtttttaccatattcattctctcattgagaaaggatttgcaccacttaaagatgcaagttacttgacaaatgggtatttggacaccgtcattgattgggttccgggaatggaaggcatccgtctcaaggatttcccgctggactggagcactgacctcaatgacaaagttttgatgttcactacagaagctcctcaaaggtcacacaaggtttcacatcatattttccacacgttcgatgagttggagcctagtattataaaaactttgtcattgaggtataatcacatttacaccatcggcccactgcaattacttcttgatcaaatacccgaagagaaaaagcaaactggaattacgagtctccatggatacagtttagtaaaagaagaaccagagtgtttccagtggcttcagtctaaagaaccaaattccgtcgtttatgtaaattttggaagtactacagtaatgtctttagaagacatgacggaatttggttggggacttgctaatagcaaccattatttcctttggatcatccgatcaaacttggtgataggggaaaatgcagttttgccccctgaacttgaggaacatataaagaaaagaggctttattgctagctggtgttcacaagaaaaggtcttgaagcacccttcggttggagggttcttgactcattgtgggtggggatcgaccatcgagagcttgtctgctggggtgccaatgatatgctggccttattcgtgggaccagctgaccaactgtaggtatatatgcaaagaatgggaggttgggctcgagatgggaaccaaagtgaaacgagatgaagtcaagaggcttgtacaagagttgatgggagaaggaggtcacaaaatgaggaacaaggctaaagattggaaagaaaaggctcgcattgcaatagctcctaacggttcatcttctttgaacatagacaaaatggtcaaggaaatcaccgtgctagcaagaaactagtcgac

SEQ ID NO: 17 - DNA, 1395 bp, synthetic construct
  source 1..1395: mol_type = other DNA
gcggccgcatggcggaacaacaaaagatcaagaaatcaccacacgttctactcatcccattccctttacaaggccatataaaccctttcatccagtttggcaaacgattaatctccaaaggtgtcaaaacaacacttgttaccaccatccacaccttaaactcaaccctaaaccacagtaacaccaccaccacctccatcgaaatccaagcaatttccgatggttgtgatgaaggcggttttatgagtgcaggagaatcatatttggaaacattcaaacaagttgggtctaaatcactagctgacttaatcaagaagcttcaaagtgaaggaaccacaattgatgcaatcatttatgattctatgactgaatgggttttagatgttgcaattgagtttggaatcgatggtggttcgtttttcactcaagcttgtgttgtaaacagcttatattatcatgttcataagggtttgatttctttgccattgggtgaaactgtttcggttcctggatttccagagcttcaacggtgggagacaccgttaattttgcagaatcatgagcaaatacagagcccttggtctcagatgttgtttggtcagtttgctaatattgatcaagcacgttgggtcttcacaaatagtttttacaagctcgaggaagaggtaatagagtggacgagaaagatatggaacttgaaggtaatcgggccaacacttccatccatgtaccttgacaaacgacttgatgatgataaagataacggatttaatctctacaaagcaaaccatcatgagtgcatgaactggttagacgataagccaaaggaatcagttgtttacgtagcatttggtagcctggtgaaacatggacccgaacaagtggaagaaatcacacgggctttaatagatagtgatgtcaacttcttgtgggttatcaaacataaagaagagggaaagctcccagaaaatctttcggaagtaataaaaaccggaaagggtttgattgtagcatggtgcaaacaattggatgtgttagcacacgaatcagtaggatgctttgttacacattgtgggttcaactcaactcttgaagcaataagtcttggagtccccgttgttgcaatgcctcaattttcggatcaaactacaaatgccaagcttctagatgaaattttgggtgttggagttagagttaaggctgatgagaatgggatagtgagaagaggaaatcttgcgtcatgtattaagatgattatggaggaggaaagaggagtaataatccgaaagaatgcggtaaaatggaaggatttggctaaagtagccgttcatgaaggtggtagctcagacaatgatattgtcgaatttgtaagtgagctaattaaggcttaattaa

SEQ ID NO: 18 - DNA, 1389 bp, synthetic construct
  source 1..1389: mol_type = other DNA
ggatccatggaaaataaaacggagaccaccgttcgccggcgccggagaataatattattcccggtaccatttcaaggccacattaacccaattcttcagctagccaatgtgttgtactctaaaggattcagtatcaccatctttcacaccaacttcaacaaacccaaaacatctaattaccctcacttcactttcagattcatcctcgacaacgacccacaagacgaacgcatttccaatctaccgactcatggtccgctcgctggtatgcggattccgattatcaacgaacacggagctgacgaattacgacgcgaactggaactgttgatgttagcttctgaagaagatgaagaggtatcgtgtttaatcacggatgctctttggtacttcgcgcaatctgttgctgacagtcttaacctccgaccgcttgttttgatgacaagcagcttgtttaattttcatgcacatgtttcacttcctcagtttgatgagcttggttacctcgatcctgatgacaaaacccgtttggaagaacaagcgagtgggtttcctatgctaaaagtgaaagacatcaagtctgcgtattcgaactggcaaatactcaaagagatattagggaagatgataaaacaaacaaaagcatcttcaggagtcatctggaactcatttaaggaactcgaagagtctgagctcgaaactgttatccgtgagatcccggctccaagtttcttgataccactccccaagcatttgacagcctcttccagcagcttactagaccacgatcgaaccgtttttcaatggttagaccaacaaccgccaagttcggtactgtatgttagttttggtagtactagtgaagtggatgagaaagatttcttggaaatagctcgtgggttggttgatagcaagcagtcgtttttatgggtggttcgacctgggtttgtcaagggttcgacgtgggtcgaaccgttgccagatgggttcttgggtgaaagaggacgtattgtgaaatgggttccacagcaagaagtgctagctcatggagcaataggcgcattctggactcatagcggatggaactctacgttggaaagcgtttgtgaaggtgttcctatgattttctcggattttgggctcgatcaaccgttgaatgctagatacatgagtgatgttttgaaggtaggggtgtatttggaaaatgggtgggaaagaggagagatagcaaatgcaataagaagagttatggtggatgaagaaggagaatacattagacagaatgcaagagttttgaaacaaaaggcagatgtttctttgatgaagggtggttcgtcttacgaatcattagagtctctagtttcttacatttcatcgttgtaagtcgac